European Patent Specification EP 3 156 423 B1, published February 19, 2025. Title: Multiple Analogous Type Antigen Peptide. Applicant: RIKEN ANIMAL ALLERGY CLINICAL LABORATORIES INC. NIPPON ZENYAKU KOGYO CO., LTD. The sequence listing filed with the application follows.

SEQUENCE LISTING (3 sequences)

SEQ ID NO: 1 - protein, 14 aa, Homo sapiens
DWIEGETYQCRVTH

SEQ ID NO: 2 - protein, 14 aa, Canis familiaris
DWIEGETYYCRVTH

SEQ ID NO: 3 - protein, 14 aa, Mus musculus
DWIEGYGYQCIVDH